European Patent Application EP 4 588 936 A1, published July 23, 2025. Title: ANTIBODIES SPECIFICALLY BINDING TO RSV. Applicant: NANJING VAZYME BIOTECH CO., LTD. Application EP 23900084.7, filed December 8, 2023. The sequence listing filed with the application follows.

SEQUENCE LISTING (44 sequences)

SEQ ID NO: 1 - protein, 8 aa, Synthetic construct
EFTFNIHA

SEQ ID NO: 2 - protein, 8 aa, Synthetic construct
ISSTGEGT

SEQ ID NO: 3 - protein, 16 aa, Synthetic construct
ARYSFRYGELRGTFDI

SEQ ID NO: 4 - protein, 6 aa, Synthetic construct
QSVGDS

SEQ ID NO: 5 - skipped

SEQ ID NO: 6 - protein, 8 aa, Synthetic construct
QQYDESWT

SEQ ID NO: 7 - protein, 123 aa, Synthetic construct
DALLLQSGGGLMQPGGSLRLSCAASEFTFNIHAMTWVRQSPGKGLEWVSGISSTGEGTYYTDSVKGRFTISRDNSKSTLYLQMNSLRAEDTATYFCARYSFRYGELRGTFDIWGQGVLVSVSS

SEQ ID NO: 8 - protein, 106 aa, Synthetic construct
DIQMTQTPSTLSASVGDRVIITCRASQSVGDSVAWFQQKPGRAPKLLIYDTTNLERGVPSRFSGSFSGTAFTLTITRLQPDDFATYYCQQYDESWTFGQGTKVEVK

SEQ ID NO: 9 - protein, 8 aa, Synthetic construct
GFSVSDYG

SEQ ID NO: 10 - protein, 8 aa, Synthetic construct
IRSHGDGT

SEQ ID NO: 11 - protein, 21 aa, Synthetic construct
ARDRVWAHDYDDTAWLDAFDL

SEQ ID NO: 12 - protein, 6 aa, Synthetic construct
QSVGSL

SEQ ID NO: 13 - skipped

SEQ ID NO: 14 - protein, 9 aa, Synthetic construct
QQYKSHSPP

SEQ ID NO: 15 - protein, 128 aa, Synthetic construct
EEQLVESGGGLVRPGGSLRLSCVASGFSVSDYGMHWVRQAPGRGLEYVSAIRSHGDGTYYVNSVKGRFIISRDNSKNTLYLQMGSLSAEDMAVYYCARDRVWAHDYDDTAWLDAFDLWGQGTTVIVSS

SEQ ID NO: 16 - protein, 107 aa, Synthetic construct
DIQMTQSPSTLSASVGDKVTITCRASQSVGSLLAWYQQKPGKAPKLLIYDASNLQRGVPSRFSGSGSGTEFTLTISSLQPDDFATYYCQQYKSHSPPFGQGTKLEIK

SEQ ID NO: 17 - protein, 8 aa, Synthetic construct
GASVSDDD

SEQ ID NO: 18 - protein, 7 aa, Synthetic construct
IDQTGSF

SEQ ID NO: 19 - protein, 19 aa, Synthetic construct
ARGGLVVTDVGQGWDAFDV

SEQ ID NO: 20 - protein, 6 aa, Synthetic construct
QDIDNW

SEQ ID NO: 21 - skipped

SEQ ID NO: 22 - protein, 9 aa, Synthetic construct
QQGDSFPLT

SEQ ID NO: 23 - protein, 125 aa, Synthetic construct
QVQLQQWGAGLLKPSETLSLTCAVDGASVSDDDWTWIRQSPGKGLEWIGQIDQTGSFNYNPSLRSRVTISPDTSKNHFSLSLTSVTAADTALYYCARGGLVVTDVGQGWDAFDVWGQGTMVTVSS

SEQ ID NO: 24 - protein, 107 aa, Synthetic construct
DIQLTQSPSSVSASVGDRITITCRASQDIDNWLAWYQQKPGEAPKLLIYAASTLQSGVPSRFSGSGAGTEFTLTITSLQPEDFAGYFCQQGDSFPLTFGGGTKVDIK

SEQ ID NO: 25 - protein, 8 aa, Synthetic construct
GYTFSDNA

SEQ ID NO: 26 - protein, 8 aa, Synthetic construct
ITANNGNT

SEQ ID NO: 27 - protein, 16 aa, Synthetic construct
AREVVNYGLGSLHFDY

SEQ ID NO: 28 - protein, 6 aa, Synthetic construct
KLGNDY

SEQ ID NO: 29 - skipped

SEQ ID NO: 30 - protein, 9 aa, Synthetic construct
QAWDGTTVI

SEQ ID NO: 31 - protein, 123 aa, Synthetic construct
QLQLVQSGTEVKKPGASVKVSCKASGYTFSDNAINWVRQAPGQGLEWLGWITANNGNTNYAQKIQGRVTMTTDTSTSTVYMELRSLGSDDTAVYYCAREVVNYGLGSLHFDYWGQGTLVTVSS

SEQ ID NO: 32 - protein, 106 aa, Synthetic construct
SYELTQPPSVSVSPGQTVSISCSGDKLGNDYASWYQQKPGQSPLLVIYEDAKRPSGIPERFSGSNSGNTATLTISGTQAMDDADYYCQAWDGTTVIFGGGTKLTVL

SEQ ID NO: 33 - protein, 107 aa, Synthetic construct
RTVAAPSVFIFPPSDEQLKSGTASVVCLLNNFYPREAKVQWKVDNALQSGNSQESVTEQDSKDSTYSLSSTLTLSKADYEKHKLYACEVTHQGLSSPVTKSFNRGEC

SEQ ID NO: 34 - protein, 106 aa, Synthetic construct
GQPKAAPSVTLFPPSSEELQANKATLVCLISDFYPGAVTVAWKADSSPVKAGVETTTPSKQSNNKYAASSYLSLTPEQWKSHRSYSCQVTHEGSTVEKTVAPTECS

SEQ ID NO: 35 - protein, 330 aa, Synthetic construct
ASTKGPSVFPLAPSSKSTSGGTAALGCLVKDYFPEPVTVSWNSGALTSGVHTFPAVLQSSGLYSLSSVVTVPSSSLGTQTYICNVNHKPSNTKVDKKVEPKSCDKTHTCPPCPAPELLGGPSVFLFPPKPKDTLYITREPEVTCVVVDVSHEDPEVKFNWYVDGVEVHNAKTKPREEQYNSTYRVVSVLTVLHQDWLNGKEYKCKVSNKALPAPIEKTISKAKGQPREPQVYTLPPSRDELTKNQVSLTCLVKGFYPSDIAVEWESNGQPENNYKTTPPVLDSDGSFFLYSKLTVDKSRWQQGNVFSCSVMHEALHNHYTQKSLSLSPGK

SEQ ID NO: 36 - DNA, 369 bp, Synthetic construct
  source 1..369: mol_type = other DNA
gatgcgctcctgttgcagtctgggggaggcctgatgcagccgggggggtccctgagactctcctgtgcagcctctgaattcactttcaacatccacgccatgacgtgggtccgccagtctcctgggaagggactggagtgggtctcaggtatcagtagcacgggtgaaggcacctattacacagactccgtgaagggccggttcaccatctccagagacaattccaagagtactctctatcttcaaatgaacagcctgcgggccgaggacacggccacatatttctgtgcgagatattcctttcggtatggggaactacggggaacatttgacatctggggccagggagtcctggtctccgtctcctca

SEQ ID NO: 37 - DNA, 318 bp, Synthetic construct
  source 1..318: mol_type = other DNA
gacatccagatgacccagactccctccactctgtctgcgtctgttggagacagagtcatcatcacttgccgggccagtcagagtgttggtgactcggtggcctggtttcagcagaaaccagggagagcccctaaactcctgatctatgacaccaccaatttagaacgtggggtcccatcaaggttcagcggcagtttctctgggacagcattcactctcaccatcaccaggttgcagcctgatgattttgcaacttattactgccaacaatatgatgaatcttggacgttcggccaagggaccaaggtggaggtcaaa

SEQ ID NO: 38 - DNA, 384 bp, Synthetic construct
  source 1..384: mol_type = other DNA
gaggagcagctggtggagtctgggggaggcttggtccggccgggtgggtctctgagactctcctgtgtagcctctggattcagtgtcagtgactatggcatgcattgggtccgccaggctccagggaggggactggaatatgtttcggccattagaagtcatggggatggcacatattatgtaaactctgtgaagggcaggttcattatctccagagacaattccaagaatacgttgtatcttcaaatgggcagcctgagcgctgaggacatggctgtctactactgtgcgagagatagagtctgggcccacgactacgatgacaccgcgtggcttgatgcttttgatctctggggccaagggacaacggtcatcgtctcttca

SEQ ID NO: 39 - DNA, 321 bp, Synthetic construct
  source 1..321: mol_type = other DNA
gacatccagatgacccagtctccttccaccctgtctgcatctgttggagacaaagtcaccatcacctgccgggccagtcagagtgttggtagcttattggcctggtatcagcagaaaccagggaaagcccctaaactcctgatctatgacgcctccaatttgcaacgtggggtcccatcaaggttcagcggcagtggatctgggacagaattcactctcaccatcagcagcctgcagcctgatgattttgcaacttattactgtcaacaatataagagtcattctccgccctttggccaggggaccaagctggagatcaaa

SEQ ID NO: 40 - DNA, 375 bp, Synthetic construct
  source 1..375: mol_type = other DNA
caggtacagttacagcagtggggcgcaggactgttgaagccttcggagaccctgtccctcacctgcgctgtcgatggtgcgtcggtcagtgatgacgactggacctggatccgccagtccccagggaagggcctagagtggattggacaaatcgatcaaactggaagcttcaattacaacccgtccctcaggagtcgagtcaccatttcaccagacacgtccaagaatcacttttccctgagtctgacttctgtgaccgccgcggacacggctctctactactgtgcgagaggcggactggtggtgactgatgtcggacagggttgggatgcttttgatgtctggggccaagggacaatggtcaccgtctcttca

SEQ ID NO: 41 - DNA, 321 bp, Synthetic construct
  source 1..321: mol_type = other DNA
gacatccagctgacccagtctccatcttccgtgtctgcatctgtgggagacagaatcaccatcacttgtcgggcgagtcaggatattgacaactggttagcctggtatcagcagaaaccaggggaagcccctaaactcctgatctatgctgcatccactttgcaaagtggggtcccatcaaggttcagcggcagtggagctgggacagaattcactctcaccatcaccagcctgcagcctgaagattttgcaggttacttttgtcaacagggtgacagtttcccgctcactttcggcggggggaccaaggtggacatcaaa

SEQ ID NO: 42 - DNA, 369 bp, Synthetic construct
  source 1..369: mol_type = other DNA
cagcttcagctggtacagtctggaacggaggtgaagaagcctggggcctcagtgaaggtctcctgcaaggcttctggttacacctttagtgacaatgctatcaactgggtgcgacaggcccctggacaagggcttgagtggttgggatggatcaccgccaacaacggaaacacaaactatgcacagaagatccagggcagagtcaccatgaccacagacacatccacgagcacggtctacatggagctgaggagcctgggctctgacgacacggccgtttattactgtgcgagggaagtggtcaactatggtttggggagtctacattttgactattggggccagggaaccctggtcaccgtctcctca

SEQ ID NO: 43 - DNA, 318 bp, Synthetic construct
  source 1..318: mol_type = other DNA
tcctacgagctgactcagccaccctcagtgtccgtgtccccaggacagacagtcagcatcagctgctctggagataaactggggaatgactatgctagttggtatcagcagaagccaggccagtcccctctgttggtcatttatgaagatgccaagcggccctcagggatccctgagcgattctctggctccaactccgggaacacagccactctgaccatcagcgggacccaggctatggatgacgctgactattactgtcaggcgtgggacggcaccactgtgattttcggcggagggaccaagctgaccgtccta

SEQ ID NO: 44 - protein, 574 aa, Synthetic construct
MELLILKANAITTILTAVTFCFASGQNITEEFYQSTCSAVSKGYLSALRTGWYTSVITIELSNIKENKCNGTDAKVKLIKQELDKYKNAVTELQLLMQSTPPTNNRARRELPRFMNYTLNNAKKTNVTLSKKRKRRFLGFLLGVGSAIASGVAVSKVLHLEGEVNKIKSALLSTNKAVVSLSNGVSVLTFKVLDLKNYIDKQLLPILNKQSCSISNIETVIEFQQKNNRLLEITREFSVNAGVTTPVSTYMLTNSELLSLINDMPITNDQKKLMSNNVQIVRQQSYSIMSIIKEEVLAYVVQLPLYGVIDTPCWKLHTSPLCTTNTKEGSNICLTRTDRGWYCDNAGSVSFFPQAETCKVQSNRVFCDTMNSLTLPSEINLCNVDIFNPKYDCKIMTSKTDVCSSVITSLGAIVSCYGKCKCTASNKNRGIIKTFSNGCDYVSNKGMDTVSVGNTLYYVNKQEGKSLYVKGEPIINFYDPLVFPSDEFDASISQVNEKINQSLAFIRKSDELLHNVNAGKSTTNIMITTIIIVIIVILLSLIAVGLLLYCKARSTPVTLSKDQLSGINNIAFSN